European Patent Application EP 4 650 443 A1, published November 19, 2025. Title: Stabilized liquid deamidase compositions. Applicant: Novozymes A/S. Application CN. The sequence listing filed with the application follows.

SEQUENCE LISTING (2 sequences)

SEQ ID NO: 1 - protein, 185 aa, Chryseobacterium sp-62563
AVSVIPNLATLNSLFAQIKNQACGTSTASSPCITFRYPVDGCYARAHKMRQILLNAGYDCEKQFVYGNLRASTGTCCVSWVYHVAILVSFKNASGVVEKRIIDPSLFSSGPVTDAAWRAACTNTSCGSASVSSFANTAGNVYYRSPSGSLLYDNNYVNTNCVLNIFSSLSGCSPSPAPSVASCGF

SEQ ID NO: 2 - protein, 109 aa, Chryseobacterium sp-62563
NQDPNLVAKESNETAMKDFGKTVPVGIEKEDGKFKISFMVTAQPYEIKDSKENAAYISMIKTAVENETPIHVFLKANTNEIAKVDKATDDDIRYFKSVFTKEVKEENRK